European Patent Application EP 4 249 510 A1, published September 27, 2023. Title: Novel formats of anti-CD28/sPD-1 fusion constructs. Applicant: Stealth IO et al. The sequence listing filed with the application follows.

SEQUENCE LISTING (73 sequences)

SEQ ID NO: 1 - protein, 111 aa, Artificial Sequence
  VL domain of anti-CD28 antibody clone 9.3
DIELTQSPASLAVSLGQRATISCRASESVEYYVTSLMQWYQQKPGQPPKLLIFAASNVESGVPARFSGSGSGTNFSLNIHPVDEDDVAMYFCQQSRKVPYTFGGGTKLEIK

SEQ ID NO: 2 - protein, 120 aa, Artificial Sequence
  VH domain of anti-CD28 antibody clone 9.3
EVKLQQSGPGLVTPSQSLSITCTVSGFSLSDYGVHWVRQSPGQGLEWLGVIWAGGGTNYNSALMSRKSISKDNSKSQVFLKMNSLQADDTAVYYCARDKGYSYYYSMDYWGQGTSVTVSS

SEQ ID NO: 3 - protein, 143 aa, Artificial Sequence
  Human wild-type soluble PD-1 protein fragment (i.e. X and/or Y)
LDSPDRPWNPPTFSPALLVVTEGDNATFTCSFSNTSESFVLNWYRMSPSNQTDKLAAFPEDRSQPGQDCRFRVTQLPNGRDFHMSVVRARRNDSGTYLCGAISLAPKAQIKESLRAELRVTERRAEVPTAHPSPSPRPAGQFQ

SEQ ID NO: 4 - protein, 143 aa, Artificial Sequence
  Mutated human soluble PD-1 protein fragment (i.e. with mutations G124S, K131Y and A132I in bold) (i.e. X and/or Y)
LDSPDRPWNPPTFSPALLVVTEGDNATFTCSFSNTSESFVLNWYRMSPSNQTDKLAAFPEDRSQPGQDCRFRVTQLPNGRDFHMSVVRARRNDSGTYLCSAISLAPYIQIKESLRAELRVTERRAEVPTAHPSPSPRPAGQFQ

SEQ ID NO: 5 - protein, 107 aa, Artificial Sequence [sequence omitted]

SEQ ID NO: 6 - protein, 328 aa, Artificial Sequence
  Human IgG1 heavy chain constant domain (CH1-hinge-CH2-CH3)
ASTKGPSVFPLAPSSKSTSGGTAALGCLVKDYFPEPVTVSWNSGALTSGVHTFPAVLQSSGLYSLSSVVTVPSSSLGTQTYICNVNHKPSNTKVDKRVEPKSCDKTHTCPPCPAPEFEGGPSVFLFPPKPKDTLMISRTPEVTCVVVDVSHEDPEVKFNWYVDGVEVHNAKTKPREEQYNSTYRVVSVLTVLHQDWLNGKEYKCKVSNKALPASIEKTISKAKGQPREPQVYTLPPSREEMTKNQVSLTCLVKGFYPSDIAVEWESNGQPENNYKTTPPVLDSDGSFFLYSKLTVDKSRWQQGNVFSCSVMHEALHNHYTQKSLSLSP

SEQ ID NO: 7 - protein, 218 aa, Artificial Sequence
  VL-CL of a bispecific protein complex of the invention (i.e. A)
DIELTQSPASLAVSLGQRATISCRASESVEYYVTSLMQWYQQKPGQPPKLLIFAASNVESGVPARFSGSGSGTNFSLNIHPVDEDDVAMYFCQQSRKVPYTFGGGTKLEIKRTVAAPSVFIFPPSDEQLKSGTASVVCLLNNFYPREAKVQWKVDNALQSGNSQESVTEQDSKDSTYSLSSTLTLSKADYEKHKVYACEVTHQGLSSPVTKSFNRGEC

SEQ ID NO: 8 - protein, 606 aa, Artificial Sequence
  Anti-CD28 heavy chain fused by linker (underlined) to wild-type soluble PD-1 fragment of a bispecific protein complex of the invention (i.e. B-C-X)
EVKLQQSGPGLVTPSQSLSITCTVSGFSLSDYGVHWVRQSPGQGLEWLGVIWAGGGTNYNSALMSRKSISKDNSKSQVFLKMNSLQADDTAVYYCARDKGYSYYYSMDYWGQGTSVTVSSASTKGPSVFPLAPSSKSTSGGTAALGCLVKDYFPEPVTVSWNSGALTSGVHTFPAVLQSSGLYSLSSVVTVPSSSLGTQTYICNVNHKPSNTKVDKRVEPKSCDKTHTCPPCPAPEFEGGPSVFLFPPKPKDTLMISRTPEVTCVVVDVSHEDPEVKFNWYVDGVEVHNAKTKPREEQYNSTYRVVSVLTVLHQDWLNGKEYKCKVSNKALPASIEKTISKAKGQPREPQVYTLPPSREEMTKNQVSLTCLVKGFYPSDIAVEWESNGQPENNYKTTPPVLDSDGSFFLYSKLTVDKSRWQQGNVFSCSVMHEALHNHYTQKSLSLSPGGGGSGGGGSGGGGSLDSPDRPWNPPTFSPALLVVTEGDNATFTCSFSNTSESFVLNWYRMSPSNQTDKLAAFPEDRSQPGQDCRFRVTQLPNGRDFHMSVVRARRNDSGTYLCGAISLAPKAQIKESLRAELRVTERRAEVPTAHPSPSPRPAGQFQ

SEQ ID NO: 9 - protein, 606 aa, Artificial Sequence
  Anti-CD28 heavy chain fused by linker (underlined) to mutated soluble PD-1 fragment of a bispecific protein complex of the invention (i.e. B-C-X)
EVKLQQSGPGLVTPSQSLSITCTVSGFSLSDYGVHWVRQSPGQGLEWLGVIWAGGGTNYNSALMSRKSISKDNSKSQVFLKMNSLQADDTAVYYCARDKGYSYYYSMDYWGQGTSVTVSSASTKGPSVFPLAPSSKSTSGGTAALGCLVKDYFPEPVTVSWNSGALTSGVHTFPAVLQSSGLYSLSSVVTVPSSSLGTQTYICNVNHKPSNTKVDKRVEPKSCDKTHTCPPCPAPEFEGGPSVFLFPPKPKDTLMISRTPEVTCVVVDVSHEDPEVKFNWYVDGVEVHNAKTKPREEQYNSTYRVVSVLTVLHQDWLNGKEYKCKVSNKALPASIEKTISKAKGQPREPQVYTLPPSREEMTKNQVSLTCLVKGFYPSDIAVEWESNGQPENNYKTTPPVLDSDGSFFLYSKLTVDKSRWQQGNVFSCSVMHEALHNHYTQKSLSLSPGGGGSGGGGSGGGGSLDSPDRPWNPPTFSPALLVVTEGDNATFTCSFSNTSESFVLNWYRMSPSNQTDKLAAFPEDRSQPGQDCRFRVTQLPNGRDFHMSVVRARRNDSGTYLCSAISLAPYIQIKESLRAELRVTERRAEVPTAHPSPSPRPAGQFQ

SEQ ID NO: 10 - protein, 147 aa, Artificial Sequence
  Human wild-type soluble PD-1 protein
FLDSPDRPWNPPTFSPALLVVTEGDNATFTCSFSNTSESFVLNWYRMSPSNQTDKLAAFPEDRSQPGQDCRFRVTQLPNGRDFHMSVVRARRNDSGTYLCGAISLAPKAQIKESLRAELRVTERRAEVPTAHPSPSPRPAGQFQTLV

SEQ ID NO: 11 - protein, 5 aa, Artificial Sequence
  H-CDR1 in Kabat of VH of clone 9.3
DYGVH

SEQ ID NO: 12 - protein, 16 aa, Artificial Sequence
  H-CDR2 in Kabat of VH of clone 9.3
VIWAGGGTNYNSALMS

SEQ ID NO: 13 - protein, 12 aa, Artificial Sequence
  H-CDR3 in Kabat of VH of clone 9.3
DKGYSYYYSMDY

SEQ ID NO: 14 - protein, 15 aa, Artificial Sequence
  L-CDR1 in Kabat of VL of clone 9.3
RASESVEYYVTSLMQ

SEQ ID NO: 15 - protein, 7 aa, Artificial Sequence
  L-CDR2 in Kabat of VL of clone 9.3
AASNVES

SEQ ID NO: 16 - protein, 9 aa, Artificial Sequence
  L-CDR3 in Kabat (or IMGT) of VL of clone 9.3
QQSRKVPYT

SEQ ID NO: 17 - protein, 8 aa, Artificial Sequence
  H-CDR1 in IMGT of VH of clone 9.3
GFSLSDYG

SEQ ID NO: 18 - protein, 7 aa, Artificial Sequence
  H-CDR2 in IMGT of VH of clone 9.3
IWAGGGT

SEQ ID NO: 19 - protein, 14 aa, Artificial Sequence
  H-CDR3 in IMGT of VH of clone 9.3
ARDKGYSYYYSMDY

SEQ ID NO: 20 - protein, 10 aa, Artificial Sequence
  L-CDR1 in IMGT of VL of clone 9.3
ESVEYYVTSL

SEQ ID NO: 21 - protein, 2 aa, Artificial Sequence
  L-CDR2 in IMGT of VL of clone 9.3
AA

SEQ ID NO: 22 - protein, 16 aa, Artificial Sequence
  H-CDR2 in Kabat of humanized VH of clone 9.3
AIWAGGGTNYASSVMG

SEQ ID NO: 23 - protein, 15 aa, Artificial Sequence
  L-CDR1 in Kabat of humanized VL of clone 9.3
RASESVEYYVTSLMA

SEQ ID NO: 24 - protein, 8 aa, Artificial Sequence
  H-CDR1 in IMGT of humanized VH of clone 9.3
GFTFSDYG

SEQ ID NO: 25 - protein, 111 aa, Artificial Sequence
  VL domain of humanized anti-CD28 antibody clone 9.3
DIVMTQSPDSLAVSLGERATINCRASESVEYYVTSLMAWYQQKPGQPPKLLIYAASNVESGVPDRFSGSGSGTNFSLTISSLQAEDVAVYYCQQSRKVPYTFGQGTKLEIK

SEQ ID NO: 26 - protein, 120 aa, Artificial Sequence
  VH domain of humanized anti-CD28 antibody clone 9.3
EVQLVQSGGGLVQPGGSLRLSCAGSGFTFSDYGVHWVRQAPGKGLEWVSAIWAGGGTNYASSVMGRFTISRDNAKNSLYLQMNSLRAEDMAVYYCARDKGYSYYYSMDYWGQGTLVTVSS

SEQ ID NO: 27 - protein, 230 aa, Artificial Sequence
  C domain (hinge-CH2-CH3 domain)
EPKSCDKTHTCPPCPAPEFEGGPSVFLFPPKPKDTLMISRTPEVTCVVVDVSHEDPEVKFNWYVDGVEVHNAKTKPREEQYNSTYRVVSVLTVLHQDWLNGKEYKCKVSNKALPASIEKTISKAKGQPREPQVYTLPPSREEMTKNQVSLTCLVKGFYPSDIAVEWESNGQPENNYKTTPPVLDSDGSFFLYSKLTVDKSRWQQGNVFSCSVMHEALHNHYTQKSLSLSP

SEQ ID NO: 28 - protein, 218 aa, Artificial Sequence
  B domain
EVKLQQSGPGLVTPSQSLSITCTVSGFSLSDYGVHWVRQSPGQGLEWLGVIWAGGGTNYNSALMSRKSISKDNSKSQVFLKMNSLQADDTAVYYCARDKGYSYYYSMDYWGQGTSVTVSSASTKGPSVFPLAPSSKSTSGGTAALGCLVKDYFPEPVTVSWNSGALTSGVHTFPAVLQSSGLYSLSSVVTVPSSSLGTQTYICNVNHKPSNTKVDKRV

SEQ ID NO: 29 - protein, 98 aa, Artificial Sequence
  CH1 domain
ASTKGPSVFPLAPSSKSTSGGTAALGCLVKDYFPEPVTVSWNSGALTSGVHTFPAVLQSSGLYSLSSVVTVPSSSLGTQTYICNVNHKPSNTKVDKRV

SEQ ID NO: 30 - protein, 218 aa, Artificial Sequence; identical to SEQ ID NO: 7
  Fc fusion construct: A) 9.3 Light Chain Kappa 9.3 VL Human Kappa constant domain

SEQ ID NO: 31 - protein, 606 aa, Artificial Sequence; identical to SEQ ID NO: 8
  Fc fusion construct with sPD-1 WT: B) 9.3 Heavy Chain IgG1-(GGGS)3 Linker- sPD1 WT 9.3 VH Human IgG1 = CH1-hinge-CH2-CH3 constant domains

SEQ ID NO: 32 - protein, 383 aa, Artificial Sequence
  Fc fusion construct with sPD-1 WT: C) Dummy Heavy Chain IgG1-(GGGS)3 Linker- sPD1 WT Human IgG1 = hinge-CH2-CH3
DKTHTCPPCPAPEFEGGPSVFLFPPKPKDTLMISRTPEVTCVVVDVSHEDPEVKFNWYVDGVEVHNAKTKPREEQYNSTYRVVSVLTVLHQDWLNGKEYKCKVSNKALPASIEKTISKAKGQPREPQVYTLPPSREEMTKNQVSLTCLVKGFYPSDIAVEWESNGQPENNYKTTPPVLDSDGSFFLYSKLTVDKSRWQQGNVFSCSVMHEALHNHYTQKSLSLSPGGGGSGGGGSGGGGSLDSPDRPWNPPTFSPALLVVTEGDNATFTCSFSNTSESFVLNWYRMSPSNQTDKLAAFPEDRSQPGQDCRFRVTQLPNGRDFHMSVVRARRNDSGTYLCGAISLAPKAQIKESLRAELRVTERRAEVPTAHPSPSPRPAGQFQ

SEQ ID NO: 33 - protein, 606 aa, Artificial Sequence; identical to SEQ ID NO: 9
  B) 9.3 Heavy Chain IgG1-(GGGS)3 Linker-sPD1 (G124S/K131Y/A132I) 9.3 VH Human IgG1 = CH1-hinge-CH2-CH3 constant domains

SEQ ID NO: 34 - protein, 383 aa, Artificial Sequence
  C) Dummy Heavy Chain IgG1-(GGGS)3 Linker- sPD1(G124S/K131Y/A132I) Human IgG1 = hinge-CH2-CH3
DKTHTCPPCPAPEFEGGPSVFLFPPKPKDTLMISRTPEVTCVVVDVSHEDPEVKFNWYVDGVEVHNAKTKPREEQYNSTYRVVSVLTVLHQDWLNGKEYKCKVSNKALPASIEKTISKAKGQPREPQVYTLPPSREEMTKNQVSLTCLVKGFYPSDIAVEWESNGQPENNYKTTPPVLDSDGSFFLYSKLTVDKSRWQQGNVFSCSVMHEALHNHYTQKSLSLSPGGGGSGGGGSGGGGSLDSPDRPWNPPTFSPALLVVTEGDNATFTCSFSNTSESFVLNWYRMSPSNQTDKLAAFPEDRSQPGQDCRFRVTQLPNGRDFHMSVVRARRNDSGTYLCSAISLAPYIQIKESLRAELRVTERRAEVPTAHPSPSPRPAGQFQ

SEQ ID NO: 35 - protein, 8 aa, Artificial Sequence
  H-CDR1 in Kabat of VH of an anti-CD28 antibody
GGSISSYY

SEQ ID NO: 36 - protein, 7 aa, Artificial Sequence
  H-CDR2 in Kabat of VH of an anti-CD28 antibody
IYYSGIT

SEQ ID NO: 37 - protein, 16 aa, Artificial Sequence
  H-CDR3 in Kabat of VH of an anti-CD28 antibody
ARWGVRRDYYYYGMDV

SEQ ID NO: 38 - protein, 7 aa, Artificial Sequence
  L-CDR1 in Kabat of VL of an anti-CD28 antibody
QSVSSSY

SEQ ID NO: 39 - protein, 3 aa, Artificial Sequence
  L-CDR2 in Kabat of VL of an anti-CD28 antibody
GAS

SEQ ID NO: 40 - protein, 9 aa, Artificial Sequence
  L-CDR3 in Kabat of VL of an anti-CD28 antibody
QQYGSSPWT

SEQ ID NO: 41 - protein, 108 aa, Artificial Sequence
  VL of an anti-CD28 antibody
EIVLTQSPGTLSLSPGERATLSCRASQSVSSSYLAWYQQKPGQAPRLLIYGASSRATGIPDRFSGSGSGTDFTLTISRLEPEDFAVYYCQQYGSSPWTFGQGTKVEIK

SEQ ID NO: 42 - protein, 122 aa, Artificial Sequence
  VH of an anti-CD28 antibody
QVQLQESGPGLVKPSETLSLTCTVSGGSISSYYWSWIRQPPGKGLEWIGYIYYSGITHYNPSLKSRVTISVDTSKIQFSLKLSSVTAADTAVYYCARWGVRRDYYYYGMDVWGQGTTVTVSS

SEQ ID NO: 43 - protein, 8 aa, Artificial Sequence
  H-CDR1 in Kabat of VH of an anti-CD28 antibody
GFTFSSYG

SEQ ID NO: 44 - protein, 8 aa, Artificial Sequence
  H-CDR1 in Kabat of VH of an anti-CD28 antibody
GFTFSRNN

SEQ ID NO: 45 - protein, 8 aa, Artificial Sequence
  H-CDR2 in Kabat of VH of an anti-CD28 antibody
ISYAGNNK

SEQ ID NO: 46 - protein, 8 aa, Artificial Sequence
  H-CDR2 in Kabat of VH of an anti-CD28 antibody
ISSNGGRT

SEQ ID NO: 47 - protein, 17 aa, Artificial Sequence
  H-CDR3 in Kabat of VH of an anti-CD28 antibody
AKDSYYDFLTDPDVLDI

SEQ ID NO: 48 - protein, 11 aa, Artificial Sequence
  H-CDR3 in Kabat of VH of an anti-CD28 antibody
TRDDELLSFDY

SEQ ID NO: 49 - protein, 6 aa, Artificial Sequence
  L-CDR1 in Kabat of VL of an anti-CD28 antibody
QSISSY

SEQ ID NO: 50 - protein, 3 aa, Artificial Sequence
  L-CDR2 in Kabat of VL of an anti-CD28 antibody
AAS

SEQ ID NO: 51 - protein, 10 aa, Artificial Sequence
  L-CDR3 in Kabat of VL of an anti-CD28 antibody
QQSYSTPPIT

SEQ ID NO: 52 - protein, 122 aa, Artificial Sequence; identical to SEQ ID NO: 42
  VH of an anti-CD28 antibody

SEQ ID NO: 53 - protein, 108 aa, Artificial Sequence; identical to SEQ ID NO: 41
  VL of an anti-CD28 antibody

SEQ ID NO: 54 - protein, 124 aa, Artificial Sequence
  VH of an anti-CD28 antibody
QVQLVESGGGVVQPGRSLRLSCAASGFTFSSYGMHWVRQAPGKGLEWVAVISYAGNNKYYADSVKGRFTVSRDNSKKTLYLQMNSLRSEDTAVYYCAKDSYYDFLTDPDVLDIWGQGTMVTVSS

SEQ ID NO: 55 - protein, 108 aa, Artificial Sequence
  VL of an anti-CD28 antibody
DIQMTQSPSSLSASVGDRVTITCRASQSISSYLNWYQQKPGKAPKLLIYAASSLQSGVPSRFSGSGSGTDFTLTISSLQPEDFATYYCQQSYSTPPITFGQGTRLEIK

SEQ ID NO: 56 - protein, 118 aa, Artificial Sequence
  VH of an anti-CD28 antibody
EVQLVESGGGLVQPGGSLRLSCAASGFTFSRNNMHWVRQAPGKGLEYVSGISSNGGRTYYADSVKGRFTISRDNSKNTLYLQMGGLRAADMAVYFCTRDDELLSFDYWGQGTLVTVSS

SEQ ID NO: 57 - protein, 8 aa, Artificial Sequence
  H-CDR1 in Kabat of VH of an anti-CD28 antibody
GYTFTSYY

SEQ ID NO: 58 - protein, 8 aa, Artificial Sequence
  H-CDR2 in Kabat of VH of an anti-CD28 antibody
IYPGNVNT

SEQ ID NO: 59 - protein, 13 aa, Artificial Sequence
  H-CDR3 in Kabat of VH of an anti-CD28 antibody
TRSHYGLDWNFDV

SEQ ID NO: 60 - protein, 6 aa, Artificial Sequence
  L-CDR1 in Kabat of VL of an anti-CD28 antibody
QNIYVW

SEQ ID NO: 61 - protein, 3 aa, Artificial Sequence
  L-CDR2 in Kabat of VL of an anti-CD28 antibody
KAS

SEQ ID NO: 62 - protein, 8 aa, Artificial Sequence
  L-CDR3 in Kabat of VL of an anti-CD28 antibody
QQGQTYPY

SEQ ID NO: 63 - protein, 107 aa, Artificial Sequence
  VL of an anti-CD28 antibody
DIQMTQSPSSLSASVGDRVTITCQASQNIYVWLNWYQQKPGKAPKLLIYKASNLHTGVPSRFSGSGSGTDFTLTISSLQPEDIATYYCQQGQTYPYTFGQGTKLEIK

SEQ ID NO: 64 - protein, 120 aa, Artificial Sequence
  VH of an anti-CD28 antibody
QVQLVQSGAEVVKPGASVKVSCKASGYTFTSYYIHWVRQAPGQGLEWIGSIYPGNVNTNYAQKFQGRATLTVDTSISTAYMELSRLRSDDTAVYYCTRSHYGLDWNFDVWGKGTTVTVSS

SEQ ID NO: 65 - protein, 5 aa, Artificial Sequence
  H-CDR1 in Kabat of VH of clone 1A7[CD28] H1L1
SYAMS

SEQ ID NO: 66 - protein, 17 aa, Artificial Sequence
  H-CDR2 in Kabat of VH of clone 1A7[CD28] H1L1
TISGSGDSTYYADSVKG

SEQ ID NO: 67 - protein, 12 aa, Artificial Sequence
  H-CDR3 in Kabat of VH of clone 1A7[CD28] H1L1
SGPGLRQVGFDY

SEQ ID NO: 68 - protein, 11 aa, Artificial Sequence
  L-CDR1 in Kabat of VL of clone 1A7[CD28] H1L1
RASQSISSYLN

SEQ ID NO: 69 - protein, 7 aa, Artificial Sequence
  L-CDR2 in Kabat of VL of clone 1A7[CD28] H1L1
AASSLQS

SEQ ID NO: 70 - protein, 9 aa, Artificial Sequence
  L-CDR3 in Kabat of VL of clone 1A7[CD28] H1L1
QQSYSTPFT

SEQ ID NO: 71 - protein, 9 aa, Artificial Sequence
  L-CDR3 in Kabat of VL of clone 1A7[CD28] H1 L1.71
QQVYSTPFT

SEQ ID NO: 72 - protein, 5 aa, Artificial Sequence
  H-CDR1 in Kabat of VH of clone 1A7[CD28] H1.1 L1.71
SYYMS

SEQ ID NO: 73 - protein, 17 aa, Artificial Sequence
  H-CDR2 in Kabat of VH of clone 1A7[CD28] H1.14 L1
TISESGDSTYYADSVKG